European Patent Application EP 4 660 296 A1, published December 10, 2025. Title: ENGINEERED STRAIN AND THE CONSTRUCTION METHOD AND USE THEREOF. Applicant: INNOBIO Co., Ltd. Application EP PCT/CN2024/142151, filed December 25, 2024. The sequence listing filed with the application follows.

SEQUENCE LISTING (10 sequences)

SEQ ID NO: 1 - protein, 485 aa, synthetic construct
MSELSQLSPQPLWDIFAKICTIPHPSYHEEQLAEYIVGWAKEKGFHVERDQVGNILIRKPATAGMENRKPVVLQAHLDMVPQKNNDTVHDFTKDPIQPYIDGEWVKARGTTLGADNGIGMASALAVLADENVVHGPLEVLLTMTEEAGMDGAFGLQGNWLQADILINTDSEEEGEIYMGCAGGIDFTSNLHLDREAVPAGFETFKLTLKGLKGGHSGGEIHVGLANANKLLVRFLAGHAEELDLRLIDFNGGTLRNAIPREAFATIAVAADKVDVLKSLVNTYQEILKNELAEKEKNLALLLDSVANDKAALIAKSRDTFIRLLNATPNGVIRNSDVAKGVVETSLNVGVVTMTDNNVEIHCLIRSLIDSGKDYVVSMLDSLGKLAGAKTEAKGAYPGWQPDANSPVMHLVRETYQRLFNKTPNIQIIHAGLECGLFKKPYPEMDMVSIGPTITGPHSPDEQVHIESVGHYWTLLTELLKEIPKK

SEQ ID NO: 2 - protein, 239 aa, synthetic construct
MVIKAQSPAGFAEEYIIESIWNNRFPPGTILPAERELSELIGATRTTLREVLQRLARDGWLTIQHGKPTKVNNFWETSGLNILETLARLDHESVPQLIDNLLSVRTNISTIFIRTAFRQHPDKAQEVLATANEVADHADTFAELDYNIFRGLAFASGNPIYGLILNGMKGIYTRIGRHYFANPEARSLALGFYHKLSALCSEGAHDQVYETVRRYGHESGEIWHRMQKNLPGDLAIQGR

SEQ ID NO: 3 - protein, 264 aa, synthetic construct
MAISIKTPEDIEKMRVAGRLAAEVLEMIEPYVKPGVSTGELDRICNDYIVNEQHAVSACLGYHGYPKSVCISINEVVCHGIPDDAKLLKDGDILNIDVTVIKDGFHGDTSKMFIVGKPTIMGERLCRITQESLYLALRMVKPGINLREIGAAIQKFVEAEGFSVVREYCGHGIGRGFHEEPNVLHYDSRETNVVLKPGMTFTIEPMVNAGKKEIRTMKDGWTVKTKDRSLSAQYEHTIVVTDNGCEILTLRKDDTIPAIISHDE

SEQ ID NO: 4 - protein, 485 aa, synthetic construct
MSELSQLSPQPLWDIFAKICSIPHPSYHEEQLAEYIVGWAKEKGFHVERDQVGNILIRKPATAGMENRKPVVLQAHLDMVPQKNNDTVHDFTKDPIQPYIDGEWVKARGTTLGADNGIGMASALAVLADENVVHGPLEVLLTMTEEAGMDGAFGLQGNWLQADILINTDSEEEGEIYMGCAGGIDFTSNLHLDREAVPAGFETFKLTLKGLKGGHSGGEIHVGLGNANKLLVRFLAGHAEELDLRLIDFNGGTLRNAIPREAFATIAVAADKVDVLKSLVNTYQEILKNELAEKEKNLALLLDSVANDKAALIAKSRDTFIRLLNATPNGVIRNSDVAKGVVETSLNVGVVTMTDNNVEIHCLIRSLIDSGKDYVVSMLDSLGKLAGAKTEAKGAYPGWQPDANSPVMHLVRETYQRLFNKTPNIQIIHAGLECGLFKKPYPEMDMVSIGPTITGPHSPDEQVHIESVGHYWTLLTELLKEIPAK

SEQ ID NO: 5 - protein, 239 aa, synthetic construct
MVIKAQSPAGFAEEYIIESIWNNRFPPGTILPAERELSELIGATRTTLREVLQRLARDGWLTIQHGKPTKVNNFWETSGLNILETLARLDHESVPQLIDNLLSVRTNISTIFIRTAFRQHPDKAQEVLATANEVADHADAFAELDYNIFRGLAFASGNPIYGLILNGMKGLYTRIGRHYFANPEARSLALGFYHKLSALCSEGAHDQVYETVRRYGHESGEIWHRMQKNLPGDLAIQGR

SEQ ID NO: 6 - protein, 264 aa, synthetic construct
MAISIKTPEDIEKMRVAGRLAAEVLEMIEPYVKPGVSTGELDRICNDYIVNEQHAVSACLGYHGYPKSVCISINEVVCHGIPDDAKLLKDGDIVNIDVTVIKDGFHGDTSKMFIVGKPTIMGERLCRITQESLYLALRMVKPGINLREIGAAIQKFVEAEGFSVVREYCGHGIGRGFHEEPQVLHYDSRETNVVLKPGMTFTIEPMVNAGKKEIRTMKDGWTVKTKDRSLSAQYEHTIVVTDNGCEILTLRKDDTIPAIISHDE

SEQ ID NO: 7 - DNA, 25 bp, synthetic construct
  source 1..25: mol_type = other DNA
gaattcatgcagggttctgtgacag

SEQ ID NO: 8 - DNA, 53 bp, synthetic construct
  source 1..53: mol_type = other DNA
cgatccgccaccgccagagccacctccgccctcgtcagcgatgcttgccggtg

SEQ ID NO: 9 - DNA, 50 bp, synthetic construct
  source 1..50: mol_type = other DNA
ggcggaggtggctctggcggtggcggatcgcatccacgttttcaaaccgc

SEQ ID NO: 10 - DNA, 25 bp, synthetic construct
  source 1..25: mol_type = other DNA
ccatggttaagcgagaagcactcgg